European Patent Specification EP 3 692 169 B1, published August 16, 2023. Title: BIOMARKERS FOR NEURODEGENERATIVE AND/OR NEUROMUSCULAR DISEASES. Applicant: Universiteit Antwerpen. The sequence listing filed with the application follows.

SEQUENCE LISTING (8 sequences)

SEQ ID NO: 1 - DNA, 21 bp, Artificial Sequence
  Fwd Primer PFN2
cggcagagctggtagagtctt

SEQ ID NO: 2 - DNA, 21 bp, Artificial Sequence
  Rev Primer PFN2
tagcagctagaacccagagtc

SEQ ID NO: 3 - DNA, 19 bp, Artificial Sequence
  Fwd Primer GAMT
tggcacacacaccagttca

SEQ ID NO: 4 - DNA, 20 bp, Artificial Sequence
  Rev Primer GAMT
aaggcgtagtagcggcagtc

SEQ ID NO: 5 - DNA, 17 bp, Artificial Sequence
  Primer 10453
atgcatcccttaagcac

SEQ ID NO: 6 - DNA, 18 bp, Artificial Sequence
  Primer 10454
ccagagggcagaactttg

SEQ ID NO: 7 - DNA, 20 bp, Artificial Sequence
  Primer oIMR8744
caaatgttgcttgtctggtg

SEQ ID NO: 8 - DNA, 20 bp, Artificial Sequence
  Primer oIMR8745
gtcagtcgagtgcacagttt